European Patent Application EP 4 656 738 A1, published December 3, 2025. Title: Composition for predicting a risk of developing liver cancer. Applicant: UIF (University Industry Foundation), Yonsei University. The sequence listing filed with the application follows.

SEQUENCE LISTING (17 sequences)

SEQ ID NO: 1 - DNA, 514 bp, Homo sapiens
  source 1..514: mol_type = genomic DNA
cgaggtaaagatcgtccagccttcataggccacctggttccgtccccctcccccagctactcgggcacgtgtcccgactcccgccagcaggccgtgggggtgatgtggccgccatgaacccaccaaggacaagtagggcctggttttagctgcaaatgcaacaagtctctccgctgagccgcagctgctaccctctgccttctgctcctccgccagggcacggccccccctgcgccccaaactgagcggcaaagtcagggcccgcggccggatgctcagagctaaaggccgcggaggacagatgtgcttcttcctccttcccgcgtctccccatacaagtactaccccgcacgtcccatcaggcttgcctgtgggccaggattcagggtcctgagccgaaacctaccaggagagagaaggctctggagacctctgtaacagtcgtgcggagaagacaaagtcagctgcgtgcgtctcctccggcgccggctctgcaaggagggaggagggggcg

SEQ ID NO: 2 - DNA, 611 bp, Homo sapiens
  source 1..611: mol_type = genomic DNA
gggcgagggaggagcctgaggagactcgcccggctcaaccccgacgtccgcgccccggccgcctgttggccatggcgggcctgggcctgggctccgccgttcccgtgtggctggccgaggacgacctcggctgcatcatctgccaggggctgctggactggcccgccacgctgccctgcggccacagcttctgccgccactgcctggaggccctgtggggcgcccgcgacgcccgccgctgggcctgccccacttgccgccagggcgccgcgcagcagccgcacctgcggaagaacacgctactgcaggacctggccgacaagtaccgccgcgccgcacgcgagatacaggcgggctccgaccctgcccactgcccctgcccgggctccagttccctctccagcgcggccgcgaggccccggcgccgcccggaactgcagcgggtagggaggccgggcccgcagctcccctggctcccccgggctgcccgccgcctgaccctttcccatgtggctcgaacccctttcctcagccgttctacttttacgttccttttctcagtctaaaagtcgagttccgctcttcggaggcactttggaaagttcataaaa

SEQ ID NO: 3 - DNA, 1300 bp, Homo sapiens
  source 1..1300: mol_type = genomic DNA
gggtgaggtcacttgctagaaccctgcgagggggcggtgccgaggcgtggaggtgatcggagtggacagagaggcggccccagaagttagtcggcgggatttgggcgcgagtgcttcccaagcgggcggggcaataggctgttccgggtgggacggaggacactggcggtctccgggacaaagacagcggttggggaagggatggatggccgggcctccaggcgtctccagactggggaaggggtagggggttaagggatcagagggcggcgtcctggccccgcaggcacgtgccgcgcccttcccccgggcccaggcccgcacccgcccgcctcccgtccgtgcaggcctcacctgggcctccagtcacgccgcagacaaggcgggctcgcgggggttcggggcgggctcgaggcccatggcccggcgactgcggcgggagcggtagagcgtccgggtgcgccctgtgcgggttgctgagagggcgcgggaggcggggtctccccggcgccccgcccccaccacctgggggagccctgccccgccccgccacctgggggagccccgcctccacggccgcgtcgggggcggtgtcgcccggaaccgcagcccccctgtttcctccccgcctcgcggcccctcagtcgcccctatttccggcgcgggacccccaccccggtacctgcacacctcatgcgcccgcagtttcgagcctgcggggctgagtcactcggcgacccgaaaattcccgccgtgaccccgcgctgcccgggcggagctccaggtggtcttgggtccgcgcccccgctccggacccccaaccctcccagccccaccccgctctcttcttcgtgtccaatcggccgccgagttacaagccactccctgatccgacttggctcccaccgcccggacccccgcccagcttcggctttgccagctcgcagtatcagcgagccgcggcctcctgtgcgaggcccacctctgcggccccagctgatcatcgggcgcacgctagggttttgcaatcccgcccccgtacccctcaccctgggacagcgctgccccctgcaaagcccggccctgccctgccctgccctgtggcttcctccctcggcctccctgcggcggccccgggctcccacggtccggagcacacagccccattgtcccggttatcggtactttgttatactgtatttgattatgcaggaccggatcggggacgcagagctccgggagggccgggctggcgtgactcagccgggtgctgcgacccagctccaactgcctttacgta

SEQ ID NO: 4 - DNA, 514 bp, synthetic construct
  misc_feature 1..514: note = Bisulfite converted Marker 1
  source 1..514: mol_type = other DNA
cgaggtaaagatcgtttagtttttataggttatttggtttcgttttttttttttagttattcgggtacgtgtttcgattttcgttagtaggtcgtgggggtgatgtggtcgttatgaatttattaaggataagtagggtttggttttagttgtaaatgtaataagttttttcgttgagtcgtagttgttattttttgttttttgttttttcgttagggtacggttttttttgcgttttaaattgagcggtaaagttagggttcgcggtcggatgtttagagttaaaggtcgcggaggatagatgtgtttttttttttttttcgcgtttttttatataagtattatttcgtacgttttattaggtttgtttgtgggttaggatttagggttttgagtcgaaatttattaggagagagaaggttttggagatttttgtaatagtcgtgcggagaagataaagttagttgcgtgcgtttttttcggcgtcggttttgtaaggagggaggagggggcg

SEQ ID NO: 5 - DNA, 611 bp, synthetic construct
  misc_feature 1..611: note = Bisulfite converted Marker 2
  source 1..611: mol_type = other DNA
gggcgagggaggagtttgaggagattcgttcggtttaatttcgacgttcgcgtttcggtcgtttgttggttatggcgggtttgggtttgggtttcgtcgttttcgtgtggttggtcgaggacgatttcggttgtattatttgttaggggttgttggattggttcgttacgttgttttgcggttatagtttttgtcgttattgtttggaggttttgtggggcgttcgcgacgttcgtcgttgggtttgttttatttgtcgttagggcgtcgcgtagtagtcgtatttgcggaagaatacgttattgtaggatttggtcgataagtatcgtcgcgtcgtacgcgagatataggcgggtttcgattttgtttattgtttttgttcgggttttagttttttttttagcgcggtcgcgaggtttcggcgtcgttcggaattgtagcgggtagggaggtcgggttcgtagtttttttggttttttcgggttgttcgtcgtttgatttttttttatgtggttcgaatttttttttttagtcgttttatttttacgtttttttttttagtttaaaagtcgagtttcgtttttcggaggtattttggaaagtttataaaa

SEQ ID NO: 6 - DNA, 1300 bp, synthetic construct
  misc_feature 1..1300: note = Bisulfite converted Marker 3
  source 1..1300: mol_type = other DNA
gggtgaggttatttgttagaattttgcgagggggcggtgtcgaggcgtggaggtgatcggagtggatagagaggcggttttagaagttagtcggcgggatttgggcgcgagtgttttttaagcgggcggggtaataggttgtttcgggtgggacggaggatattggcggttttcgggataaagatagcggttggggaagggatggatggtcgggtttttaggcgtttttagattggggaaggggtagggggttaagggattagagggcggcgttttggtttcgtaggtacgtgtcgcgtttttttttcgggtttaggttcgtattcgttcgtttttcgttcgtgtaggttttatttgggtttttagttacgtcgtagataaggcgggttcgcgggggttcggggcgggttcgaggtttatggttcggcgattgcggcgggagcggtagagcgttcgggtgcgttttgtgcgggttgttgagagggcgcgggaggcggggttttttcggcgtttcgtttttattatttgggggagttttgtttcgtttcgttatttgggggagtttcgtttttacggtcgcgtcgggggcggtgtcgttcggaatcgtagtttttttgtttttttttcgtttcgcggttttttagtcgtttttattttcggcgcgggatttttatttcggtatttgtatattttatgcgttcgtagtttcgagtttgcggggttgagttattcggcgattcgaaaattttcgtcgtgatttcgcgttgttcgggcggagttttaggtggttttgggttcgcgttttcgtttcggatttttaatttttttagttttatttcgttttttttttcgtgtttaatcggtcgtcgagttataagttattttttgattcgatttggtttttatcgttcggattttcgtttagtttcggttttgttagttcgtagtattagcgagtcgcggttttttgtgcgaggtttatttttgcggttttagttgattatcgggcgtacgttagggttttgtaatttcgttttcgtattttttattttgggatagcgttgttttttgtaaagttcggttttgttttgttttgttttgtggttttttttttcggtttttttgcggcggtttcgggtttttacggttcggagtatatagttttattgtttcggttatcggtattttgttatattgtatttgattatgtaggatcggatcggggacgtagagtttcgggagggtcgggttggcgtgatttagtcgggtgttgcgatttagttttaattgtttttacgta

SEQ ID NO: 7 - DNA, 20 bp, synthetic construct
  misc_feature 1..20: note = Methylated Forward Primer for Marker 1
  source 1..20: mol_type = other DNA
aaccgacgccgaaaaaaacg

SEQ ID NO: 8 - DNA, 26 bp, synthetic construct
  misc_feature 1..26: note = Methylated Reverse Primer for Marker 1
  source 1..26: mol_type = other DNA
gaaggttttggagatttttgtaatag

SEQ ID NO: 9 - DNA, 26 bp, synthetic construct
  misc_feature 1..26: note = Unmethylated Forward Primer for Marker 1
  source 1..26: mol_type = other DNA
ttacaaaaccaacaccaaaaaaaaca

SEQ ID NO: 10 - DNA, 28 bp, synthetic construct
  misc_feature 1..28: note = Methylated Forward Primer for marker 1
  source 1..28: mol_type = other DNA
gagaaggttttggagatttttgtaatag

SEQ ID NO: 11 - DNA, 21 bp, synthetic construct
  misc_feature 1..21: note = Methylated Reverse Primer for marker 1
  source 1..21: mol_type = other DNA
ctccttacaaaaccgacgccg

SEQ ID NO: 12 - DNA, 20 bp, synthetic construct
  misc_feature 1..20: note = Unmethylated Reverse Primer for marker 1
  source 1..20: mol_type = other DNA
tccttacaaaaccaacacca

SEQ ID NO: 13 - DNA, 25 bp, synthetic construct
  misc_feature 1..25: note = Methylated Forward Primer for Marker 2
  source 1..25: mol_type = other DNA
ttatggcgggtttgggtttgggttt

SEQ ID NO: 14 - DNA, 24 bp, synthetic construct
  misc_feature 1..24: note = Methylated Reverse Primer for Marker 2
  source 1..24: mol_type = other DNA
caacccctaacaaataatacaacc

SEQ ID NO: 15 - DNA, 22 bp, synthetic construct
  misc_feature 1..22: note = Methylated Forward Primer for Marker 3
  source 1..22: mol_type = other DNA
ggattagggagtggtttgtaat

SEQ ID NO: 16 - DNA, 18 bp, synthetic construct
  misc_feature 1..18: note = Methylated Reverse Primer for Marker 3
  source 1..18: mol_type = other DNA
cccgctctcttcttcgta

SEQ ID NO: 17 - DNA, 20 bp, synthetic construct
  misc_feature 1..20: note = Unmethylated Reverse Primer for Marker 3
  source 1..20: mol_type = other DNA
accccactctcttcttcata